European Patent Specification EP 3 889 611 B1, published May 27, 2026. Title: COMPOSITIONS AND METHODS FOR PERFORMING METHYLATION DETECTION ASSAYS. Applicant: Exact Sciences Development Company, LLC. Application EP. The sequence listing filed with the application follows.

SEQUENCE LISTING (62 sequences)

SEQ ID NO: 1 - DNA, 48 bp, Artificial sequence
  DNA primer/probe
tccctcgcgcgtggcttccgccttctgcgcggctggggtgcccggtgg

SEQ ID NO: 2 - DNA, 26 bp, Artificial sequence
  DNA primer/probe
gcgggacactccgaaggcgcaaggag

SEQ ID NO: 3 - DNA, 44 bp, Artificial sequence
  DNA primer/probe
ggcctgctgaaaatgactgaatataaacttgtggtagttggagc

SEQ ID NO: 4 - DNA, 46 bp, Artificial sequence
  DNA primer/probe
ctctattgttggatcatattcgtccacaaaatgattctgaattagc

SEQ ID NO: 5 - DNA, 21 bp, Artificial sequence
  DNA primer/probe
cggttttcgttcgttttttcg

SEQ ID NO: 6 - DNA, 20 bp, Artificial sequence
  DNA primer/probe
gtaacttccgccttctacgc

SEQ ID NO: 7 - DNA, 18 bp, Artificial sequence
  DNA primer/probe
cgccgagggttcgtttat

SEQ ID NO: 8 - DNA, 23 bp, Artificial sequence
  DNA primer/probe
gtttaattttcggtttcgtcgtc

SEQ ID NO: 9 - DNA, 17 bp, Artificial sequence
  DNA primer/probe
ctcccgacgtcgctacg

SEQ ID NO: 10 - DNA, 20 bp, Artificial sequence
  DNA primer/probe
cgccgaggcggttttttgcg

SEQ ID NO: 11 - DNA, 18 bp, Artificial sequence
  DNA primer/probe
cttgtggtagttggagca

SEQ ID NO: 12 - DNA, 20 bp, Artificial sequence
  DNA primer/probe
gcgcgtccagtggcgtaggc

SEQ ID NO: 13 - DNA, 22 bp, Artificial sequence
  DNA primer/probe
aaacttgtggtagttggacctt

SEQ ID NO: 14 - DNA, 20 bp, Artificial sequence
  DNA primer/probe
gcgcgtcctgtggcgtaggc

SEQ ID NO: 15 - DNA, 25 bp, Artificial sequence
  DNA primer/probe
tataaacttgtggtagttggacctc

SEQ ID NO: 16 - DNA, 20 bp, Artificial sequence
  DNA primer/probe
gcgcgtcccgtggcgtaggc

SEQ ID NO: 17 - DNA, 21 bp, Artificial sequence
  DNA primer/probe
acttgtggtagttggagctca

SEQ ID NO: 18 - DNA, 20 bp, Artificial sequence
  DNA primer/probe
gcgcgtccatggcgtaggca

SEQ ID NO: 19 - DNA, 21 bp, Artificial sequence
  DNA primer/probe
acttgtggtagttggagctct

SEQ ID NO: 20 - DNA, 20 bp, Artificial sequence
  DNA primer/probe
gcgcgtccttggcgtaggca

SEQ ID NO: 21 - DNA, 22 bp, Artificial sequence
  DNA primer/probe
aacttgtggtagttggagatgc

SEQ ID NO: 22 - DNA, 20 bp, Artificial sequence
  DNA primer/probe
gcgcgtccctggcgtaggca

SEQ ID NO: 23 - DNA, 18 bp, Artificial sequence
  DNA primer/probe
ggtagttggagctggtca

SEQ ID NO: 24 - DNA, 20 bp, Artificial sequence
  DNA primer/probe
gcgcgtccacgtaggcaaga

SEQ ID NO: 25 - DNA, 22 bp, Artificial sequence
  DNA primer/probe
ctattgttggatcatattcgtc

SEQ ID NO: 26 - DNA, 70 bp, Homo sapiens
ggggccggggccgacagcccacgctggcgcggcaggcgcgtgcgcccgccgttttcgtgagcccgagcag

SEQ ID NO: 27 - DNA, 70 bp, Homo sapiens
ggggtcggggtcgatagtttacgttggcgcggtaggcgcgtgcgttcgtcgttttcgtgagttcgagtag

SEQ ID NO: 28 - DNA, 12 bp, Artificial sequence
  DNA primer/probe
gttggcgcggta

SEQ ID NO: 29 - DNA, 20 bp, Artificial sequence
  DNA primer/probe
gtcggggtcgatagtttacg

SEQ ID NO: 30 - DNA, 20 bp, Artificial sequence
  DNA primer/probe
cgaactcacgaaaacgacga

SEQ ID NO: 31 - DNA, 12 bp, Artificial sequence
  DNA primer/probe
gacgaacgcacg

SEQ ID NO: 32 - DNA, 19 bp, Artificial sequence
  DNA primer/probe
actcgaactcacgaaaacg

SEQ ID NO: 33 - DNA, 70 bp, Homo sapiens
ggggucggggucgauaguuuacgutggcgcgguaggcgcgtgcguucgucgttttcgtgaguucgaguag

SEQ ID NO: 34 - DNA, 21 bp, Artificial sequence
  DNA primer/probe
gacgcggaggttggcgcggta

SEQ ID NO: 35 - DNA, 21 bp, Artificial sequence
  DNA primer/probe
gacgcggaggacgaacgcacg

SEQ ID NO: 36 - DNA, 28 bp, Artificial sequence
  DNA primer/probe
ctcgggctcacgaaaacggcgggcgcac

SEQ ID NO: 37 - DNA, 77 bp, Homo sapiens
tctctgtgtactaatttccctttttggccggacgtggtggctcacgcctgtaatcccagcactttgggaggccaaag

SEQ ID NO: 38 - DNA, 77 bp, Homo sapiens
tttttgtgtattaatttttttttttggtcggacgtggtggtttacgtttgtaattttagtattttgggaggttaaag

SEQ ID NO: 39 - DNA, 12 bp, Artificial sequence
  DNA primer/probe
acgtggtggttt

SEQ ID NO: 40 - DNA, 28 bp, Artificial sequence
  DNA primer/probe
tgtgtattaatttttttttttggtcgga

SEQ ID NO: 41 - DNA, 28 bp, Artificial sequence
  DNA primer/probe
cctcccaaaatactaaaattacaaacgt

SEQ ID NO: 42 - DNA, 21 bp, Artificial sequence
  DNA primer/probe
gacgcggagacgtggtggttt

SEQ ID NO: 43 - DNA, 35 bp, Artificial sequence
  DNA primer/probe
gtgctgggattacaggcgtgagccaccacgtccgg

SEQ ID NO: 44 - DNA, 77 bp, Homo sapiens
ccatctatagaaaaatggattagggccgggcacagtggctcacgcctgtaatcccagcactttgggaggccgaggca

SEQ ID NO: 45 - DNA, 77 bp, Homo sapiens
ttatttatagaaaaatggattagggtcgggtatagtggtttacgtttgtaattttagtattttgggaggtcgaggta

SEQ ID NO: 46 - DNA, 12 bp, Artificial sequence
  DNA primer/probe
aacgtaaaccac

SEQ ID NO: 47 - DNA, 22 bp, Artificial sequence
  DNA primer/probe
gaaaaatggattagggtcgggt

SEQ ID NO: 48 - DNA, 28 bp, Artificial sequence
  DNA primer/probe
tcgacctcccaaaatactaaaattacaa

SEQ ID NO: 49 - DNA, 21 bp, Artificial sequence
  DNA primer/probe
gacgcggagaacgtaaaccac

SEQ ID NO: 50 - DNA, 36 bp, Artificial sequence
  DNA primer/probe
cggcctcccaaagtgctgggattacaggcgtgagcc

SEQ ID NO: 51 - DNA, 29 bp, Artificial sequence
  DNA primer/probe
agccggttttccggctgagactccgcgtc

SEQ ID NO: 52 - DNA, 27 bp, Artificial sequence
  DNA primer/probe
tttgtttttttgattaggtgtttaaga

SEQ ID NO: 53 - skipped
  DNA primer/probe

SEQ ID NO: 54 - skipped
  DNA primer/probe

SEQ ID NO: 55 - skipped
  DNA primer/probe

SEQ ID NO: 56 - skipped
  DNA primer/probe

SEQ ID NO: 57 - skipped
  DNA primer/probe

SEQ ID NO: 58 - skipped
  DNA primer/probe

SEQ ID NO: 59 - DNA, 21 bp, Artificial sequence
  DNA primer/probe
caccaacctcataaccttatc

SEQ ID NO: 60 - DNA, 21 bp, Artificial sequence
  DNA primer/probe
ccacggacgatagtgttgtgg

SEQ ID NO: 61 - DNA, 166 bp, Homo sapiens
ctctgcaggttctatttgctttttcccagatgagctctttttctggtgtttgtctctctgactaggtgtctaagacagtgttgtgggtgtaggtactaacactggctcgtgtgacaaggccatgaggctggtgtaaagcggccttggagtgtgtattaagtaggtg

SEQ ID NO: 62 - DNA, 166 bp, Homo sapiens
ttttgtaggttttatttgtttttttttagatgagttttttttttggtgtttgtttttttgattaggtgtttaagatagtgttgtgggtgtaggtattaatattggtttgtgtgataaggttatgaggttggtgtaaagtggttttggagtgtgtattaagtaggtg